European Patent Specification EP 3 595 615 B1, published January 10, 2024. Title: Treatment for gingivitis. Applicant: The University of Melbourne. Application PCT/AU2018/050231. The sequence listing filed with the application follows.

SEQUENCE LISTING (12 sequences)

SEQ ID NO: 1 - protein, 21 aa, Artificial Sequence
  Phosphopetide
  MOD_RES (6)..(6): PHOSPHORYLATION
  MOD_RES (8)..(10): PHOSPHORYLATION
  MOD_RES (17)..(17): PHOSPHORYLATION
QMEAESISSSEEIVPNSVEQK

SEQ ID NO: 2 - protein, 25 aa, Artificial Sequence
  Phosphopeptide
  MOD_RES (15)..(15): PHOSPHORYLATION
  MOD_RES (17)..(19): PHOSPHORYLATION
RELEELNVPGEIVESLSSSEESITR

SEQ ID NO: 3 - protein, 25 aa, Artificial Sequence
  Phosphopeptide
  MOD_RES (11)..(13): PHOSPHORYLATION
  MOD_RES (16)..(16): PHOSPHORYLATION
NANEEEYSIGSSSEESAEVATEEVK

SEQ ID NO: 4 - protein, 21 aa, Artificial Sequence
  Phosphopeptide
  MOD_RES (8)..(10): PHOSPHORYLATION
  MOD_RES (16)..(16): PHOSPHORYLATION
KNTMEHVSSSEESIISQETYK

SEQ ID NO: 5 - DNA, 17 bp, Artificial Sequence
  Forward primer
gtgccagcmgccgcggt

SEQ ID NO: 6 - DNA, 19 bp, Artificial Sequence
  Reverse primer
ggactachvgggtwtctaa

SEQ ID NO: 7 - DNA, 18 bp, Artificial Sequence
  Probe sequence
actccagactttcctgac

SEQ ID NO: 8 - DNA, 18 bp, Artificial Sequence
  Probe sequence
agacgcaatcccctcctt

SEQ ID NO: 9 - DNA, 20 bp, Artificial Sequence
  Probe sequence
actctgccgaccattcttct

SEQ ID NO: 10 - DNA, 21 bp, Artificial Sequence
  Probe sequence
agagatagagtttctcttcgg

SEQ ID NO: 11 - DNA, 20 bp, Artificial Sequence
  Probe sequence
cggttatccagaagaagggg

SEQ ID NO: 12 - DNA, 21 bp, Artificial Sequence
  Probe sequence
ctaatgggacgcaaagctctc